European Patent Application EP 4 417 616 A1, published August 21, 2024. Title: LXR ANTAGONISTS. Applicant: Ospedale San Raffaele S.r.l. The sequence listing filed with the application follows.

SEQUENCE LISTING (12 sequences)

SEQ ID NO: 1 - DNA, 21 bp, synthetic construct
  source 1..21: mol_type = other DNA
acatcatccctgcctctactg

SEQ ID NO: 2 - DNA, 20 bp, synthetic construct
  source 1..20: mol_type = other DNA
accacctggtgctcagtgta

SEQ ID NO: 3 - DNA, 19 bp, synthetic construct
  source 1..19: mol_type = other DNA
ccaggccagtacggaattc

SEQ ID NO: 4 - DNA, 19 bp, synthetic construct
  source 1..19: mol_type = other DNA
cctcgccaaaccagtagga

SEQ ID NO: 5 - DNA, 14 bp, synthetic construct
  source 1..14: mol_type = other DNA
ggcgggcgcagatc

SEQ ID NO: 6 - DNA, 24 bp, synthetic construct
  source 1..24: mol_type = other DNA
ttgttgataagctgaagcatgtct

SEQ ID NO: 7 - DNA, 19 bp, synthetic construct
  source 1..19: mol_type = other DNA
acagcggggaatgggtact

SEQ ID NO: 8 - DNA, 20 bp, synthetic construct
  source 1..20: mol_type = other DNA
gactggtacaacgagcggat

SEQ ID NO: 9 - DNA, 30 bp, synthetic construct
  source 1..30: mol_type = other DNA
ttcagaaacacatgctgatcctcataattc

SEQ ID NO: 10 - DNA, 30 bp, synthetic construct
  source 1..30: mol_type = other DNA
attaagcaccacagcatatcgcaagaaagt

SEQ ID NO: 11 - protein, 8 aa, synthetic construct
SIINFEKL

SEQ ID NO: 12 - protein, 17 aa, synthetic construct
ISQAVHAAHAEINEAGR